European Patent Specification EP 4 010 007 B1, published November 15, 2023. Title: Production of MHC II/CII complexes. Applicant: Fraunhofer-Gesellschaft zur Förderung der angewandten Forschung e.V. The sequence listing filed with the application follows.

SEQUENCE LISTING (34 sequences)

SEQ ID NO: 1 - protein, 11 aa, Homo sapiens
  CII peptide 261-271
AGFKGEQGPKG

SEQ ID NO: 2 - protein, 11 aa, Homo sapiens
  CII peptide 261-271, Lys = Xaa
  UNSURE 10: Xaa = any proteinogenic amino acids except Lys; preferably Xaa = Arg, Ala, Gly or Gln
AGFKGEQGPXG

SEQ ID NO: 3 - protein, 11 aa, Artificial Sequence
  CII peptide 261-271; Gln = Xaa
  UNSURE 7: Xaa = any proteinogenic amion acid except Gln; preferably Xaa = Ala, Arg, His or Gly
AGFKGEXGPKG

SEQ ID NO: 4 - protein, 11 aa, Artificial Sequence
  CII peptide 261-271; Glu = Xaa
  UNSURE 6: Xaa = any proteinogenic amino acid except Glu, preferably Xaa = Ala, Asp, Gln or Gly
AGFKGXQGPKG

SEQ ID NO: 5 - protein, 11 aa, Artificial Sequence
  CII peptide 261-271; Gly = Xaa
  UNSURE 5: Xaa = any proteinogenic amino acid expect Gly; preferably Xaa = Ala, Ser, Val or Leu
AGFKXEQGPKG

SEQ ID NO: 6 - protein, 11 aa, Artificial Sequence
  CII peptide 261-271; Gln = Xaa and Lys = Xaa
  UNSURE 7: Xaa = any proteinogenic amino acid expect Gln; preferably Xaa = Ala, Arg, His or Gly
  UNSURE 10: Xaa = any proteinogenic amino acid except Lys; preferably Xaa = Arg, Ala, Gly or Gln
AGFKGEXGPXG

SEQ ID NO: 7 - protein, 11 aa, Artificial Sequence
  CII peptide 261-271; Glu = Xaa and Lys = Xaa
  UNSURE 6: Xaa = any proteinogenic amino acid except Glu; preferably Xaa = Ala, Asp, Gln or Gly
  UNSURE 10: Xaa = any proteinogenic amino acid expect Lys, preferably Xaa = Arg, Ala, Gly or Gln
AGFKGXQGPXG

SEQ ID NO: 8 - protein, 11 aa, Artificial Sequence
  CII peptide 261-271; Gly = Xaa and Lys = Xaa
  UNSURE 5: Xaa = any proteinogenic amino acid except Gly; preferably Xaa = Ala, Ser, Val or Leu
AGFKXEQGPXG

SEQ ID NO: 9 - protein, 11 aa, Artificial Sequence
  CII peptide 261-271; Lys = Arg
AGFKGEQGPRG

SEQ ID NO: 10 - protein, 13 aa, Homo sapiens
  CII peptide 261-273
AGFKGEQGPKGEP

SEQ ID NO: 11 - protein, 13 aa, Artificial Sequence
  CII peptide 261-273; Lys = Xaa
  UNSURE 10: Xaa = any proteinogenic amino acid except Lys; preferably Lys = Arg, Ala, Gly or Gln
AGFKGEQGPXGEP

SEQ ID NO: 12 - protein, 13 aa, Artificial Sequence
  CII peptide 261-273; Lys = Arg
AGFKGEQGPRGEP

SEQ ID NO: 13 - protein, 15 aa, Homo sapiens
  CII peptide 259-273
GIAGFKGEQGPKGEP

SEQ ID NO: 14 - protein, 15 aa, Artificial Sequence
  CII peptide 259-273; Lys = Xaa
  UNSURE 12: Xaa = any proteinogenic amino acid; preferably Xaa = Arg, Ala, Gly or Gln
GIAGFKGEQGPXGEP

SEQ ID NO: 15 - protein, 15 aa, Artificial Sequence
  CII peptide 259-273; Lys = Arg
GIAGFKGEQGPRGEP

SEQ ID NO: 16 - protein, 275 aa, Artificial Sequence
  DR4 construct alpha-chain
MKLCILLAVVAFVGLSLGIKEEHVIIQAEFYLNPDQSGEFMFDFDGDEIFHVDMAKKETVWRLEEFGRFASFEAQGALANIAVDKANLEIMTKRSNYTPITNVPPEVTVLTNSPVELREPNVLICFIDKFTPPVVNVTWLRNGKPVTTGVSETVFLPREDHLFRKFHYLPFLPSTEDVYDCRVEHWGLDEPLLKHWEFDASGGGENLYFQGGGGSLTDTLQAETDQLEDEKSALQTEIANLLKEKEKLEFILAAHGGGGSGLNDIFEAQKIEWHE

SEQ ID NO: 17 - protein, 311 aa, Artificial Sequence
  DR4 construct beta-chain with hCII259-273 peptide
MKLCILLAVVAFVGLSLGSAWSHPQFEKGIAGFKGEQGPKGEPSGGGSLVPRGSGGGGSGDTRPRFLEQVKHECHFFNGTERVRFLDRYFYHQEEYVRFDSDVGEYRAVTELGRPDAEYWNSQKDLLEQKRAAVDTYCRHNYGVGESFTVQRRVYPEVTVYPAKTQPLQHHNLLVCSVNGFYPGSIEVRWFRNGQEEKTGVVSTGLIQNGDWTFQTLVMLETVPRSGEVYTCQVEHPSLTSPLTVEWRARSGGGENLYFQGGGGSRIARLEEKVKTLKAQNSELASTANMLREQVAQLKQKVMNHHHHHHH

SEQ ID NO: 18 - protein, 248 aa, Artificial Sequence
  Minimal DR4 construct alpha-chain
MKLCILLAVVAFVGLSLGIKEEHVIIQAEFYLNPDQSGEFMFDFDGDEIFHVDMAKKETVWRLEEFGRFASFEAQGALANIAVDKANLEIMTKRSNYTPITNVPPEVTVLTNSPVELREPNVLICFIDKFTPPVVNVTWLRNGKPVTTGVSETVFLPREDHLFRKFHYLPFLPSTEDVYDCRVEHWGLDEPLLKHWEFDASGGGGGGSLTDTLQAETDQLEDEKSALQTEIANLLKEKEKLEFILAAH

SEQ ID NO: 19 - protein, 288 aa, Artificial Sequence
  Minimal DR4 construct beta-chain with hCII259-273 peptide
MKLCILLAVVAFVGLSLGGIAGFKGEQGPKGEPSGGGSGGGGSGDTRPRFLEQVKHECHFFNGTERVRFLDRYFYHQEEYVRFDSDVGEYRAVTELGRPDAEYWNSQKDLLEQKRAAVDTYCRHNYGVGESFTVQRRVYPEVTVYPAKTQPLQHHNLLVCSVNGFYPGSIEVRWFRNGQEEKTGVVSTGLIQNGDWTFQTLVMLETVPRSGEVYTCQVEHPSLTSPLTVEWRARSGGGGGGSRIARLEEKVKTLKAQNSELASTANMLREQVAQLKQKVMNHHHHHHH

SEQ ID NO: 20 - protein, 311 aa, Artificial Sequence
  DR4 construct beta-chain with hCLIPmut
MKLCILLAVVAFVGLSLGSAWSHPQFEKPVSKARMATGALAQASGGGSLVPRGSGGGGSGDTRPRFLEQVKHECHFFNGTERVRFLDRYFYHQEEYVRFDSDVGEYRAVTELGRPDAEYWNSQKDLLEQKRAAVDTYCRHNYGVGESFTVQRRVYPEVTVYPAKTQPLQHHNLLVCSVNGFYPGSIEVRWFRNGQEEKTGVVSTGLIQNGDWTFQTLVMLETVPRSGEVYTCQVEHPSLTSPLTVEWRARSGGGENLYFQGGGGSRIARLEEKVKTLKAQNSELASTANMLREQVAQLKQKVMNHHHHHHH

SEQ ID NO: 21 - protein, 290 aa, Artificial Sequence
  Aq construct alpha-chain
MKLCILLAVVAFVGLSLGEDDIEADHVGFYGIVVYQSPGDIGQYTHEFDGDEWFYVDLDKKETVWMLPEFGQLTSFDPQGGLQNIATGKHNLGGWTKRSNFTPATNEAPQATVFPKSPVLLGQPNTLICFVDNIFPPVINITWLRNSKSVTDGVYETSFLVNRDHSFHKLSYLTFIPSDDDIYDCKVEHWGLDEPVLKHWEPEIPATMSELTETVSGGGENLYFQGGGGSLTDTLQAETDQLEDEKSALQTEIANLLKEKEKLEFILAAHGGGGSGLNDIFEAQKIEWHE

SEQ ID NO: 22 - protein, 316 aa, Artificial Sequence
  Aq construct beta-chain with rat CII259-273 peptide
MKLCILLAVVAFVGLSLGSAWSHPQFEKGIAGFKGEQGPKGETSGGGSLVPRGSGGGGSERHFVAQLKGECYFTNGTQRIRSVNRYIYNREEWVRFDSDVGEYRAVTELGRPDAEYWNSQPEILERTRAEVDTVCRHNYEGVETHTSLRRLEQPNVAISLSRTEALNHHNTLVCSVTDFYPAKIKVRWFRNGQEETVGVSSTQLIRNGDWTFQVLVMLEMTPHQGEVYTCHVEHPSLKSPITVEWRAQSESARSKSGGGENLYFQGGGGSRIARLEEKVKTLKAQNSELASTANMLREQVAQLKQKVMNHHHHHHH

SEQ ID NO: 23 - protein, 310 aa, Artificial Sequence
  Aq construct beta-chain with rat CII259-273 peptide without His-tag
MKLCILLAVVAFVGLSLGSAWSHPQFEKGIAGFKGEQGPKGETSGGGSLVPRGSGGGGSERHFVAQLKGECYFTNGTQRIRSVNRYIYNREEWVRFDSDVGEYRAVTELGRPDAEYWNSQPEILERTRAEVDTVCRHNYEGVETHTSLRRLEQPNVAISLSRTEALNHHNTLVCSVTDFYPAKIKVRWFRNGQEETVGVSSTQLIRNGDWTFQVLVMLEMTPHQGEVYTCHVEHPSLKSPITVEWRAQSESARSKSGGGENLYFQGGGGSRIARLEEKVKTLKAQNSELASTANMLREQVAQLKQKVMNH

SEQ ID NO: 24 - protein, 316 aa, Artificial Sequence
  Aq construct beta-chain with mCLIP peptide
MKLCILLAVVAFVGLSLGSAWSHPQFEKPVSQARMATPLLMRPSGGGSLVPRGSGGGGSERHFVAQLKGECYFTNGTQRIRSVNRYIYNREEWVRFDSDVGEYRAVTELGRPDAEYWNSQPEILERTRAEVDTVCRHNYEGVETHTSLRRLEQPNVAISLSRTEALNHHNTLVCSVTDFYPAKIKVRWFRNGQEETVGVSSTQLIRNGDWTFQVLVMLEMTPHQGEVYTCHVEHPSLKSPITVEWRAQSESARSKSGGGENLYFQGGGGSRIARLEEKVKTLKAQNSELASTANMLREQVAQLKQKVMNHHHHHHH

SEQ ID NO: 25 - protein, 310 aa, Artificial Sequence
  Aq construct beta-chain with mCLIP peptide without His-tag
MKLCILLAVVAFVGLSLGSAWSHPQFEKPVSQARMATPLLMRPSGGGSLVPRGSGGGGSERHFVAQLKGECYFTNGTQRIRSVNRYIYNREEWVRFDSDVGEYRAVTELGRPDAEYWNSQPEILERTRAEVDTVCRHNYEGVETHTSLRRLEQPNVAISLSRTEALNHHNTLVCSVTDFYPAKIKVRWFRNGQEETVGVSSTQLIRNGDWTFQVLVMLEMTPHQGEVYTCHVEHPSLKSPITVEWRAQSESARSKSGGGENLYFQGGGGSRIARLEEKVKTLKAQNSELASTANMLREQVAQLKQKVMNH

SEQ ID NO: 26 - protein, 40 aa, Homo sapiens
  cFos domain
LTDTLQAETDQLEDEKSALQTEIANLLKEKEKLEFILAAH

SEQ ID NO: 27 - protein, 40 aa, Homo sapiens
  cJun domain
RIARLEEKVKTLKAQNSELASTANMLREQVAQLKQKVMNH

SEQ ID NO: 28 - protein, 15 aa, Homo sapiens
  mutated human CLIP-peptide
PVSKARMATGALAQA

SEQ ID NO: 29 - protein, 15 aa, Homo sapiens
  rat CII-peptide 259-273
GIAGFKGEQGPKGET

SEQ ID NO: 30 - protein, 10 aa, Artificial Sequence
  streptavidin-tag
SAWSHPQFEK

SEQ ID NO: 31 - protein, 11 aa, Artificial Sequence
  Chondroitin-binding peptide
EKRIWFPYRRF

SEQ ID NO: 32 - protein, 11 aa, Artificial Sequence
  chondroitin-binding peptide
YKTNFRRYYRF

SEQ ID NO: 33 - protein, 11 aa, Artificial Sequence
  chondroitin-binding peptide
VLIRHFRKRYY

SEQ ID NO: 34 - protein, 30 aa, Artificial Sequence
  hCII259-273 with N-terminal and C-terminal sequence
SAWSHPQFEKGIAGFKGEQGPKGEPSGGGS